European Patent Application EP 4 563 585 A1, published June 4, 2025. Title: METHOD FOR SITE-DIRECTED SYNTHESIS OF PROTEIN-ACTIVE MOLECULE CONJUGATE. Applicant: Nanjing GenScript Biotech Co.,Ltd. Application CN. The sequence listing filed with the application follows.

SEQUENCE LISTING (10 sequences)

SEQ ID NO: 1 - DNA, 16 bp, unidentified
  source 1..16: mol_type = other DNA
  modified_base 1: mod_base = OTHER; note = PCbt
  modified_base 16: mod_base = OTHER; note = am
acaacatatagcgcag

SEQ ID NO: 2 - protein, 397 aa, Protein
MHHHHHHKIEEGKLVIWINGDKGYNGLAEVGKKFEKDTGIKVTVEHPDKLEEKFPQVAATGDGPDIIFWAHDRFGGYAQSGLLAEITPDKAFQDKLYPFTWDAVRYNGKLIAYPIAVEALSLIYNKDLLPNPPKTWEEIPALDKELKAKGKSALMFNLQEPYFTWPLIAADGGYAFKYENGKYDIKDVGVDNAGAKAGLTFLVDLIKNKHMNADTDYSIAEAAFNKGETAMTINGPWAWSNIDTSKVNYGVTVLPTFKGQPSKPFVGVLSAGINAASPNKELAKEFLENYLLTDEGLEAVNKDKPLGAVALKSYEEELVKDPRIAATMENAQKGEIMPNIPQMSAFWYAVRTAVINAASGRQTVDEALKDAQTNSSSNNNNNNNNNNLGIEGRISHM

SEQ ID NO: 3 - protein, 245 aa, Protein
MHHHHHHVSKGEELFTGVVPILVELDGDVNGHKFSVSGEGEGDATYGKLTLKFICTTGKLPVPWPTLVTTLTYGVQCFSRYPDHMKQHDFFKSAMPEGYVQERTIFFKDDGNYKTRAEVKFEGDTLVNRIELKGIDFKEDGNILGHKLEYNYNSHNVYIMADKQKNGIKVNFKIRHNIEDGSVQLADHYQQNTPIGDGPVLLPDNHYLSTQSALSKDPNEKRDHMVLLEFVTAAGITLGMDELYK

SEQ ID NO: 4 - protein, 82 aa, Protein
MHHHHHHQIFVKTLTGKTITLEVEPSDTIENVKAKIQDKEGIPPDQQRLIFAGKQLEDGRTLSDYNIQKESTLHLVLRLRGG

SEQ ID NO: 5 - protein, 108 aa, Protein
MHHHHHHMSDSEVNQEAKPEVKPEVKPETHINLKVSDGSSEIFFKIKKTTPLRRLMEAFAKRQGKEMDSLRFLYDGIRIQADQTPEDLDMEDNDIIEAHREQIGGATY

SEQ ID NO: 6 - DNA, 65 bp, synthetic construct
  source 1..65: mol_type = other DNA
  modified_base 1: mod_base = OTHER; note = PCbt
  modified_base 65: mod_base = OTHER; note = am
aggcgaactgttttggtcataacccgctactgattgttcgcacggagtgctgtgcttgtgtaagg

SEQ ID NO: 7 - protein, 456 aa, Protein
MHHHHHHQVQLKQSGPGLVQPSQSLSITCTVSGFSLTNYGVHWVRQSPGKGLEWLGVIWSGGNTDYNTPFTSRLSINKDNSKSQVFFKMNSLQSNDTAIYYCARALTYYDYEFAYWGQGTLVTVSAASTKGPSVFPLAPSSKSTSGGTAALGCLVKDYFPEPVTVSWNSGALTSGVHTFPAVLQSSGLYSLSSVVTVPSSSLGTQTYICNVNHKPSNTKVDKKVEPKSCDKTHTCPPCPAPELLGGPSVFLFPPKPKDTLMISRTPEVTCVVVDVSHEDPEVKFNWYVDGVEVHNAKTKPREEQYNSTYRVVSVLTVLHQDWLNGKEYKCKVSNKALPAPIEKTISKAKGQPREPQVYTLPPSRDELTKNQVSLTCLVKGFYPSDIAVEWESNGQPENNYKTTPPVLDSDGSFFLYSKLTVDKSRWQQGNVFSCSVMHEALHNHYTQKSLSLSPGK

SEQ ID NO: 8 - protein, 214 aa, Protein
DILLTQSPVILSVSPGERVSFSCRASQSIGTNIHWYQQRTNGSPRLLIKYASESISGIPSRFSGSGSGTDFTLSINSVESEDIADYYCQQNNNWPTTFGAGTKLELKRTVAAPSVFIFPPSDEQLKSGTASVVCLLNNFYPREAKVQWKVDNALQSGNSQESVTEQDSKDSTYSLSSTLTLSKADYEKHKVYACEVTHQGLSSPVTKSFNRGEC

SEQ ID NO: 9 - protein, 457 aa, Protein
MHHHHHHEVQLVESGGGLVQPGGSLRLSCAASGFNIKDTYIHWVRQAPGKGLEWVARIYPTNGYTRYADSVKGRFTISADTSKNTAYLQMNSLRAEDTAVYYCSRWGGDGFYAMDYWGQGTLVTVSSASTKGPSVFPLAPSSKSTSGGTAALGCLVKDYFPEPVTVSWNSGALTSGVHTFPAVLQSSGLYSLSSVVTVPSSSLGTQTYICNVNHKPSNTKVDKKVEPKSCDKTHTCPPCPAPELLGGPSVFLFPPKPKDTLMISRTPEVTCVVVDVSHEDPEVKFNWYVDGVEVHNAKTKPREEQYNSTYRVVSVLTVLHQDWLNGKEYKCKVSNKALPAPIEKTISKAKGQPREPQVYTLPPSREEMTKNQVSLTCLVKGFYPSDIAVEWESNGQPENNYKTTPPVLDSDGSFFLYSKLTVDKSRWQQGNVFSCSVMHEALHNHYTQKSLSLSPGK

SEQ ID NO: 10 - protein, 214 aa, Protein
DIQMTQSPSSLSASVGDRVTITCRASQDVNTAVAWYQQKPGKAPKLLIYSASFLYSGVPSRFSGSRSGTDFTLTISSLQPEDFATYYCQQHYTTPPTFGQGTKVEIKRTVAAPSVFIFPPSDEQLKSGTASVVCLLNNFYPREAKVQWKVDNALQSGNSQESVTEQDSKDSTYSLSSTLTLSKADYEKHKVYACEVTHQGLSSPVTKSFNRGEC